European Patent Application EP 4 269 563 A2, published November 1, 2023. Title: Anti-GD2 Antibodies. Applicant: Memorial Sloan-Kettering Cancer Center. The sequence listing filed with the application follows.

SEQUENCE LISTING (24 sequences)

SEQ ID NO: 1 - protein, 449 aa, synthetic construct
  source 1..449: note = Chimeric 3F8 heavy chain gamma 1
QVQLKESGPGLVAPSQSLSITCTVSGFSVTNYGVHWVRQPPGKGLEWLGVIWAGGITNYNSAFMSRLSISKDNSKSQVFLKMNSLQIDDTAMYYCASRGGHYGYALDYWGQGTSVTVSSASTKGPSVFPLAPSSKSTSGGTAALGCLVKDYFPEPVTVSWNSGALTSGVHTFPAVLQSSGLYSLSSVVTVPSSSLGTQTYICNVNHKPSNTKVDKRVEPKSCDKTHTCPPCPAPELLGGPSVFLFPPKPKDTLMISRTPEVTCVVVDVSHEDPEVKFNWYVDGVEVHNAKTKPREEQYNSTYRVVSVLTVLHQDWLNGKEYKCKVSNKALPAPIEKTISKAKGQPREPQVYTLPPSRDELTKNQVSLTCLVKGFYPSDIAVEWESNGQPENNYKTTPPVLDSDGSFFLYSKLTVDKSRWQQGNVFSCSVMHEALHNHYTQKSLSLSPGK

SEQ ID NO: 2 - protein, 211 aa, synthetic construct
  source 1..211: note = Chimeric 3F8 light chain kappa
SIVMTQTPKFLLVSAGDRVTITCKASQSVSNDVTWYQQKAGQSPKLLIYSASNRYSGVPDRFTGSGYGTAFTFTISTVQAEDLAVYFCQQDYSSFGGGTKLEIKRTVAAPSVFIFPPSDEQLKSGTASVVCLLNNFYPREAKVQWKVDNALQSGNSQESVTEQDSKDSTYSLSSTLTLSKADYEKHKVYACEVTHQGLSSPVTKSFNRGEC

SEQ ID NO: 3 - protein, 446 aa, synthetic construct
  source 1..446: note = Chimeric 3F8 heavy chain gamma 4
QVQLKESGPGLVAPSQSLSITCTVSGFSVTNYGVHWVRQPPGKGLEWLGVIWAGGITNYNSAFMSRLSISKDNSKSQVFLKMNSLQIDDTAMYYCASRGGHYGYALDYWGQGTSVTVSSASTKGPSVFPLAPCSRSTSESTAALGCLVKDYFPEPVTVSWNSGALTSGVHTFPAVLQSSGLYSLSSVVTVPSSSLGTKTYTCNVDHKPSNTKVDKRVESKYGPPCPSCPAPEFLGGPSVFLFPPKPKDTLMISRTPEVTCVVVDVSQEDPEVQFNWYVDGVEVHNAKTKPREEQFNSTYRVVSVLTVLHQDWLNGKEYKCKVSNKGLPSSIEKTISKAKGQPREPQVYTLPPSQEEMTKNQVSLTCLVKGFYPSDIAVEWESNGQPENNYKTTPPVLDSDGSFFLYSRLTVDKSRWQEGNVFSCSVMHEALHNHYTQKSLSLSLGK

SEQ ID NO: 4 - protein, 448 aa, synthetic construct
  source 1..448: note = huH1 - gamma 1
QVQLVESGPGVVQPGRSLRISCAVSGFSVTNYGVHWVRQPPGKGLEWLGVIWAGGITNYNSAFMSRLTISKDNSKNTVYLQMNSLRAEDTAMYYCASRGGHYGYALDYWGQGTLVTVSSASTKGPSVFPLAPSSKSTSGGTAALGCLVKDYFPEPVTVSWNSGALTSGVHTFPAVLQSSGLYSLSSVVTVPSSSLGTQTYICNVNHKPSNTKVDKRVEPKSCDKTHTCPPCPAPELLGGPSVFLFPPKPKDTLMISRTPEVTCVVVDVSHEDPEVKFNWYVDGVEVHNAKTKPREEQYNSTYRVVSVLTVLHQDWLNGKEYKCKVSNKALPAPIEKTISKAKGQPREPQVYTLPPSRDELTKNQVSLTCLVKGFYPSDIAVEWESNGQPENNYKTTPPVLDSDGSFFLYSKLTVDKSRWQQGNVFSCSVMHEALHNHYTQKSLSLSPG

SEQ ID NO: 5 - protein, 211 aa, synthetic construct
  source 1..211: note = HuL1- kappa
EIVMTQTPATLSVSAGERVTITCKASQSVSNDVTWYQQKPGQAPRLLIYSASNRYSGVPARFSGSGYGTEFTFTISSVQSEDFAVYFCQQDYSSFGQGTKLEIKRTVAAPSVFIFPPSDEQLKSGTASVVCLLNNFYPREAKVQWKVDNALQSGNSQESVTEQDSKDSTYSLSSTLTLSKADYEKHKVYACEVTHQGLSSPVTKSFNRGEC

SEQ ID NO: 6 - protein, 448 aa, synthetic construct
  source 1..448: note = huH2 - gamma 1
QVQLKESGPGVVQPGQSLSISCAVSGFSVTNYGVHWVRQPPGKGLEWLGVIWAGGITNYNSAFMSRLTISKDNSKSTVYLKMNSLQAEDTAMYYCASRGGHYGYALDYWGQGTLVTVSSASTKGPSVFPLAPSSKSTSGGTAALGCLVKDYFPEPVTVSWNSGALTSGVHTFPAVLQSSGLYSLSSVVTVPSSSLGTQTYICNVNHKPSNTKVDKRVEPKSCDKTHTCPPCPAPELLGGPSVFLFPPKPKDTLMISRTPEVTCVVVDVSHEDPEVKFNWYVDGVEVHNAKTKPREEQYNSTYRVVSVLTVLHQDWLNGKEYKCKVSNKALPAPIEKTISKAKGQPREPQVYTLPPSRDELTKNQVSLTCLVKGFYPSDIAVEWESNGQPENNYKTTPPVLDSDGSFFLYSKLTVDKSRWQQGNVFSCSVMHEALHNHYTQKSLSLSPG

SEQ ID NO: 7 - protein, 211 aa, synthetic construct
  source 1..211: note = huL2 - kappa
SIVMTQTPKTLSVSAGERVTITCKASQSVSNDVTWYQQKPGQSPKLLIYSASNRYSGVPDRFSGSGYGTAFTFTISSVQAEDFAVYFCQQDYSSFGQGTKLEIKRTVAAPSVFIFPPSDEQLKSGTASVVCLLNNFYPREAKVQWKVDNALQSGNSQESVTEQDSKDSTYSLSSTLTLSKADYEKHKVYACEVTHQGLSSPVTKSFNRGEC

SEQ ID NO: 8 - protein, 446 aa, synthetic construct
  source 1..446: note = huH1-gamma 4
QVQLVESGPGVVQPGRSLRISCAVSGFSVTNYGVHWVRQPPGKGLEWLGVIWAGGITNYNSAFMSRLTISKDNSKNTVYLQMNSLRAEDTAMYYCASRGGHYGYALDYWGQGTLVTVSSASTKGPSVFPLAPCSRSTSESTAALGCLVKDYFPEPVTVSWNSGALTSGVHTFPAVLQSSGLYSLSSVVTVPSSSLGTKTYTCNVDHKPSNTKVDKRVESKYGPPCPSCPAPEFLGGPSVFLFPPKPKDTLMISRTPEVTCVVVDVSQEDPEVQFNWYVDGVEVHNAKTKPREEQFNSTYRVVSVLTVLHQDWLNGKEYKCKVSNKGLPSSIEKTISKAKGQPREPQVYTLPPSQEEMTKNQVSLTCLVKGFYPSDIAVEWESNGQPENNYKTTPPVLDSDGSFFLYSRLTVDKSRWQEGNVFSCSVMHEALHNHYTQKSLSLSLGK

SEQ ID NO: 9 - protein, 449 aa, synthetic construct
  source 1..449: note = huH3-gamma 1, with stability enhanced mutations
QVQLVESGPGLVQPGRSLRLTCAVSGFSVTNYGVHWVRQPPGKGLEWLGVIWAGGITNYNSAFMSRLTISKDNSKNTVYLQMNSLRAEDTAVYYCASRGGHYGYALDYWGQGTLVTVSSASTKGPSVFPLAPSSKSTSGGTAALGCLVKDYFPEPVTVSWNSGALTSGVHTFPAVLQSSGLYSLSSVVTVPSSSLGTQTYICNVNHKPSNTKVDKRVEPKSCDKTHTCPPCPAPELLGGPSVFLFPPKPKDTLMISRTPEVTCVVVDVSHEDPEVKFNWYVDGVEVHNAKTKPREEQYNSTYRVVSVLTVLHQDWLNGKEYKCKVSNKALPAPIEKTISKAKGQPREPQVYTLPPSRDELTKNQVSLTCLVKGFYPSDIAVEWESNGQPENNYKTTPPVLDSDGSFFLYSKLTVDKSRWQQGNVFSCSVMHEALHNHYTQKSLSLSPGK

SEQ ID NO: 10 - protein, 211 aa, synthetic construct
  source 1..211: note = HuL3 - kappa
SIVMTQTPAFLLVSAGERVTITCRASQSVSNDVTWYQQKAGQAPRLLIYSASNRYTGIPARFSGSGYGTEFTFTISSVQSEDFAVYFCQQDYSSFGGGTKLEIKRTVAAPSVFIFPPSDEQLKSGTASVVCLLNNFYPREAKVQWKVDNALQSGNSQESVTEQDSKDSTYSLSSTLTLSKADYEKHKVYACEVTHQGLSSPVTKSFNRGEC

SEQ ID NO: 11 - DNA, 684 bp, synthetic construct
  source 1..684: mol_type = other DNA; note = Hu3F8-H1L1-IgG1, light chain
atgggctggtcctgcatcatcctgttcctggtggccaccgccaccggcgagatcgtgatgacccagacccccgccaccctgtccgtgtccgccggcgagcgggtgaccatcacctgcaaggcctcccagtccgtgtccaacgacgtgacctggtaccagcagaagcccggccaggccccccggctgctgatctactccgcctccaaccggtactccggcgtgcccgcccggttctccggctccggctacggcaccgagttcaccttcaccatctcctccgtgcagtccgaggacttcgccgtgtacttctgccagcaggactactcctccttcggccagggcaccaagctggagatcaagcggaccgtggccgccccctccgtgttcatcttccccccctccgacgagcagctgaagtccggcaccgcctccgtggtgtgcctgctgaacaacttctacccccgggaggccaaggtgcagtggaaggtggacaacgccctgcagtccggcaactcccaggagtccgtgaccgagcaggactccaaggactccacctactccctgtcctccaccctgaccctgtccaaggccgactacgagaagcacaaggtgtacgcctgcgaggtgacccaccagggcctgtcctcccccgtgaccaagtccttcaaccggggcgagtgctag

SEQ ID NO: 12 - DNA, 1398 bp, synthetic construct
  source 1..1398: mol_type = other DNA; note = Hu3F8-H1L1-IgG1, heavy chain
atgggctggtcctgcatcatcctgttcctggtggccaccgccaccggccaggtgcagctggtggagtccggccccggcgtggtgcagcccggccggtccctgcggatctcctgcgccgtgtccggcttctccgtgaccaactacggcgtgcactgggtgcggcagccccccggcaagggcctggagtggctgggcgtgatctgggccggcggcatcaccaactacaactccgccttcatgtcccggctgaccatctccaaggacaactccaagaacaccgtgtacctgcagatgaactccctgcgggccgaggacaccgccatgtactactgcgcctcccggggcggccactacggctacgccctggactactggggccagggcaccctggtgaccgtgtcctccgcctccaccaagggcccatcggtcttccccctggcaccctcctccaagagcacctctgggggcacagcggccctgggctgcctggtcaaggactacttccccgaaccggtgacggtgtcgtggaactcaggcgccctgaccagcggcgtgcacaccttcccggccgtcctacagtcctcaggactctactccctcagcagcgtggtgaccgtgccctccagcagcttgggcacccagacctacatctgcaacgtgaatcacaagcccagcaacaccaaggtggacaagagagttgagcccaaatcttgtgacaaaactcacacatgcccaccgtgcccagcacctgaactcctggggggaccgtcagtcttcctcttccccccaaaacccaaggacaccctcatgatctcccggacccctgaggtcacatgcgtggtggtggacgtgagccacgaagaccctgaggtcaagttcaactggtacgtggacggcgtggaggtgcataatgccaagacaaagccgcgggaggagcagtacaacagcacgtaccgtgtggtcagcgtcctcaccgtcctgcaccaggactggctgaatggcaaggagtacaagtgcaaggtctccaacaaagccctcccagcccccatcgagaaaaccatctccaaagccaaagggcagccccgagaaccacaggtgtacaccctgcccccatcccgggatgagctgaccaagaaccaggtcagcctgacctgcctggtcaaaggcttctatcccagcgacatcgccgtggagtgggagagcaatgggcagccggagaacaactacaagaccacgcctcccgtgctggactccgacggctccttcttcctctacagcaagctcaccgtggacaagagcaggtggcagcaggggaacgtcttctcatgctccgtgatgcatgaggctctgcacaaccactacacgcagaagagcctctccctgtctccgggtaaatga

SEQ ID NO: 13 - DNA, 684 bp, synthetic construct; identical to SEQ ID NO: 11
  source 1..684: mol_type = other DNA; note = Hu3F8-H1L1-IgG4 light chain

SEQ ID NO: 14 - DNA, 1389 bp, synthetic construct
  source 1..1389: mol_type = other DNA; note = Hu3F8-H1L1-IgG4 heavy chain
atgggctggtcctgcatcatcctgttcctggtggccaccgccaccggccaggtgcagctggtggagtccggccccggcgtggtgcagcccggccggtccctgcggatctcctgcgccgtgtccggcttctccgtgaccaactacggcgtgcactgggtgcggcagccccccggcaagggcctggagtggctgggcgtgatctgggccggcggcatcaccaactacaactccgccttcatgtcccggctgaccatctccaaggacaactccaagaacaccgtgtacctgcagatgaactccctgcgggccgaggacaccgccatgtactactgcgcctcccggggcggccactacggctacgccctggactactggggccagggcaccctggtgaccgtgtcctccgcctccaccaagggcccctccgtgttccccctggccccctgctcccggtccacctccgagtccaccgccgccctgggctgcctggtgaaggactacttccccgagcccgtgaccgtgtcctggaactccggcgccctgacctccggcgtgcacaccttccccgccgtgctgcagtcctccggcctgtactccctgtcctccgtggtgaccgtgccctcctcctccctgggcaccaagacctacacctgcaacgtggaccacaagccctccaacaccaaggtggacaagcgggtggagtccaagtacggccccccctgcccctcctgccccgcccccgagttcctgggcggcccctccgtgttcctgttcccccccaagcccaaggacaccctgatgatctcccggacccccgaggtgacctgcgtggtggtggacgtgtcccaggaggaccccgaggtgcagttcaactggtacgtggacggcgtggaggtgcacaacgccaagaccaagccccgggaggagcagttcaactccacctaccgggtggtgtccgtgctgaccgtgctgcaccaggactggctgaacggcaaggagtacaagtgcaaggtgtccaacaagggcctgccctcctccatcgagaagaccatctccaaggccaagggccagccccgggagccccaggtgtacaccctgcccccctcccaggaggagatgaccaagaaccaggtgtccctgacctgcctggtgaagggcttctacccctccgacatcgccgtggagtgggagtccaacggccagcccgagaacaactacaagaccaccccccccgtgctggactccgacggctccttcttcctgtactcccggctgaccgtggacaagtcccggtggcaggagggcaacgtgttctcctgctccgtgatgcacgaggccctgcacaaccactacacccagaagtccctgtccctgtccctgggcaagtga

SEQ ID NO: 15 - DNA, 684 bp, synthetic construct
  source 1..684: mol_type = other DNA; note = Hu3F8-H2L2-IgG1 light chain
atgggctggtcctgcatcatcctgttcctggtggccaccgccaccggctccatcgtgatgacccagacccccaagaccctgtccgtgtccgccggcgagcgggtgaccatcacctgcaaggcctcccagtccgtgtccaacgacgtgacctggtaccagcagaagcccggccagtcccccaagctgctgatctactccgcctccaaccggtactccggcgtgcccgaccggttctccggctccggctacggcaccgccttcaccttcaccatctcctccgtgcaggccgaggacttcgccgtgtacttctgccagcaggactactcctccttcggccagggcaccaagctggagatcaagcggaccgtggccgccccctccgtgttcatcttccccccctccgacgagcagctgaagtccggcaccgcctccgtggtgtgcctgctgaacaacttctacccccgggaggccaaggtgcagtggaaggtggacaacgccctgcagtccggcaactcccaggagtccgtgaccgagcaggactccaaggactccacctactccctgtcctccaccctgaccctgtccaaggccgactacgagaagcacaaggtgtacgcctgcgaggtgacccaccagggcctgtcctcccccgtgaccaagtccttcaaccggggcgagtgctag

SEQ ID NO: 16 - DNA, 1398 bp, synthetic construct
  source 1..1398: mol_type = other DNA; note = Hu3F8-H2L2-IgG1, heavy chain
atgggctggtcctgcatcatcctgttcctggtggccaccgccaccggccaggtgcagctgaaggagtccggccccggcgtggtgcagcccggccagtccctgtccatctcctgcgccgtgtccggcttctccgtgaccaactacggcgtgcactgggtgcggcagccccccggcaagggcctggagtggctgggcgtgatctgggccggcggcatcaccaactacaactccgccttcatgtcccggctgaccatctccaaggacaactccaagtccaccgtgtacctgaagatgaactccctgcaggccgaggacaccgccatgtactactgcgcctcccggggcggccactacggctacgccctggactactggggccagggcaccctggtgaccgtgtcctccgcctccaccaagggcccatcggtcttccccctggcaccctcctccaagagcacctctgggggcacagcggccctgggctgcctggtcaaggactacttccccgaaccggtgacggtgtcgtggaactcaggcgccctgaccagcggcgtgcacaccttcccggccgtcctacagtcctcaggactctactccctcagcagcgtggtgaccgtgccctccagcagcttgggcacccagacctacatctgcaacgtgaatcacaagcccagcaacaccaaggtggacaagagagttgagcccaaatcttgtgacaaaactcacacatgcccaccgtgcccagcacctgaactcctggggggaccgtcagtcttcctcttccccccaaaacccaaggacaccctcatgatctcccggacccctgaggtcacatgcgtggtggtggacgtgagccacgaagaccctgaggtcaagttcaactggtacgtggacggcgtggaggtgcataatgccaagacaaagccgcgggaggagcagtacaacagcacgtaccgtgtggtcagcgtcctcaccgtcctgcaccaggactggctgaatggcaaggagtacaagtgcaaggtctccaacaaagccctcccagcccccatcgagaaaaccatctccaaagccaaagggcagccccgagaaccacaggtgtacaccctgcccccatcccgggatgagctgaccaagaaccaggtcagcctgacctgcctggtcaaaggcttctatcccagcgacatcgccgtggagtgggagagcaatgggcagccggagaacaactacaagaccacgcctcccgtgctggactccgacggctccttcttcctctacagcaagctcaccgtggacaagagcaggtggcagcaggggaacgtcttctcatgctccgtgatgcatgaggctctgcacaaccactacacgcagaagagcctctccctgtctccgggtaaatga

SEQ ID NO: 17 - DNA, 684 bp, synthetic construct
  source 1..684: mol_type = other DNA; note = ch3F8-IgG1, light chain
atgggctggtcctgcatcatcctgttcctggtggccaccgccaccggcagtattgtgatgacccagactcccaaattcctgcttgtatcagcaggagacagggttaccataacctgcaaggccagtcagagtgtgagtaatgatgtaacttggtaccaacagaaggcagggcagtctcctaaactgctgatatactctgcatccaatcgctattctggagtccctgaccgcttcactggcagtggatatgggacggctttcactttcaccatcagcactgtgcaggctgaagacctggcagtttatttctgtcagcaggattatagttcgttcggaggggggaccaagctggaaataaagcggaccgtggccgccccctccgtgttcatcttccccccctccgacgagcagctgaagtccggcaccgcctccgtggtgtgcctgctgaacaacttctacccccgggaggccaaggtgcagtggaaggtggacaacgccctgcagtccggcaactcccaggagtccgtgaccgagcaggactccaaggactccacctactccctgtcctccaccctgaccctgtccaaggccgactacgagaagcacaaggtgtacgcctgcgaggtgacccaccagggcctgtcctcccccgtgaccaagtccttcaaccggggcgagtgctag

SEQ ID NO: 18 - DNA, 1395 bp, synthetic construct
  source 1..1395: mol_type = other DNA; note = ch3F8-IgG1, heavy chain
atgggctggtcctgcatcatcctgttcctggtggccaccgccaccggccaggtgcagctgaaggagtcagggcctggcctggtggcgccctcacagagcctgtccatcacttgcactgtctctgggttttcagtaaccaattatggtgtacactgggttcgccagcctccaggaaagggtctggagtggctgggagtaatatgggctggtggaattacaaattataattcggctttcatgtccagactgagcatcagcaaagacaactccaagagtcaagttttcttaaaaatgaacagtctgcaaattgatgacacagccatgtactactgtgccagtcgggggggtcactacggctatgctttggactactggggtcaaggaacctcagtcaccgtctcctcagcctccaccaagggcccatcggtcttccccctggcaccctcctccaagagcacctctgggggcacagcggccctgggctgcctggtcaaggactacttccccgaaccggtgacggtgtcgtggaactcaggcgccctgaccagcggcgtgcacaccttcccggccgtcctacagtcctcaggactctactccctcagcagcgtggtgaccgtgccctccagcagcttgggcacccagacctacatctgcaacgtgaatcacaagcccagcaacaccaaggtggacaagagagttgagcccaaatcttgtgacaaaactcacacatgcccaccgtgcccagcacctgaactcctggggggaccgtcagtcttcctcttccccccaaaacccaaggacaccctcatgatctcccggacccctgaggtcacatgcgtggtggtggacgtgagccacgaagaccctgaggtcaagttcaactggtacgtggacggcgtggaggtgcataatgccaagacaaagccgcgggaggagcagtacaacagcacgtaccgtgtggtcagcgtcctcaccgtcctgcaccaggactggctgaatggcaaggagtacaagtgcaaggtctccaacaaagccctcccagcccccatcgagaaaaccatctccaaagccaaagggcagccccgagaaccacaggtgtacaccctgcccccatcccgggatgagctgaccaagaaccaggtcagcctgacctgcctggtcaaaggcttctatcccagcgacatcgccgtggagtgggagagcaatgggcagccggagaacaactacaagaccacgcctcccgtgctggactccgacggctccttcttcctctacagcaagctcaccgtggacaagagcaggtggcagcaggggaacgtcttctcatgctccgtgatgcatgaggctctgcacaaccactacacgcagaagagcctctccctgtctccgggtaaa

SEQ ID NO: 19 - DNA, 684 bp, synthetic construct; identical to SEQ ID NO: 17
  source 1..684: mol_type = other DNA; note = ch3F8-IgG4 light chain

SEQ ID NO: 20 - DNA, 1386 bp, synthetic construct
  source 1..1386: mol_type = other DNA; note = ch3F8-IgG4 heavy chain
atgggctggtcctgcatcatcctgttcctggtggccaccgccaccggccaggtgcagctgaaggagtcagggcctggcctggtggcgccctcacagagcctgtccatcacttgcactgtctctgggttttcagtaaccaattatggtgtacactgggttcgccagcctccaggaaagggtctggagtggctgggagtaatatgggctggtggaattacaaattataattcggctttcatgtccagactgagcatcagcaaagacaactccaagagtcaagttttcttaaaaatgaacagtctgcaaattgatgacacagccatgtactactgtgccagtcgggggggtcactacggctatgctttggactactggggtcaaggaacctcagtcaccgtctcctcagcctccaccaagggcccctccgtgttccccctggccccctgctcccggtccacctccgagtccaccgccgccctgggctgcctggtgaaggactacttccccgagcccgtgaccgtgtcctggaactccggcgccctgacctccggcgtgcacaccttccccgccgtgctgcagtcctccggcctgtactccctgtcctccgtggtgaccgtgccctcctcctccctgggcaccaagacctacacctgcaacgtggaccacaagccctccaacaccaaggtggacaagcgggtggagtccaagtacggccccccctgcccctcctgccccgcccccgagttcctgggcggcccctccgtgttcctgttcccccccaagcccaaggacaccctgatgatctcccggacccccgaggtgacctgcgtggtggtggacgtgtcccaggaggaccccgaggtgcagttcaactggtacgtggacggcgtggaggtgcacaacgccaagaccaagccccgggaggagcagttcaactccacctaccgggtggtgtccgtgctgaccgtgctgcaccaggactggctgaacggcaaggagtacaagtgcaaggtgtccaacaagggcctgccctcctccatcgagaagaccatctccaaggccaagggccagccccgggagccccaggtgtacaccctgcccccctcccaggaggagatgaccaagaaccaggtgtccctgacctgcctggtgaagggcttctacccctccgacatcgccgtggagtgggagtccaacggccagcccgagaacaactacaagaccaccccccccgtgctggactccgacggctccttcttcctgtactcccggctgaccgtggacaagtcccggtggcaggagggcaacgtgttctcctgctccgtgatgcacgaggccctgcacaaccactacacccagaagtccctgtccctgtccctgggcaag

SEQ ID NO: 21 - DNA, 684 bp, synthetic construct
  source 1..684: mol_type = other DNA; note = hu3F8-H3L3 light chain
atgggctggtcctgcatcatcctgttcctggtggccaccgccaccggctctatcgtcatgactcagacccctgccttcctgctggtgtccgctggagagcgtgtcactatcacttgtcgtgcctcacagagcgtgtctaacgacgtgacatggtaccagcagaaggccggtcaggctcccagactgctgatctactctgcaagtaataggtatactggcattcctgcccggttctcaggctccggatatgggaccgagttcacctttacaatctccagcgtgcagagcgaagattttgctgtctatttttgccagcaggattattcatcattcggcggcggtactaaactggaaattaagcgcaccgtggccgccccctccgtgttcatcttccccccctccgacgagcagctgaagtccggcaccgcctccgtggtgtgcctgctgaacaacttctacccccgggaggccaaggtgcagtggaaggtggacaacgccctgcagtccggcaactcccaggagtccgtgaccgagcaggactccaaggactccacctactccctgtcctccaccctgaccctgtccaaggccgactacgagaagcacaaggtgtacgcctgcgaggtgacccaccagggcctgtcctcccccgtgaccaagtccttcaaccggggcgagtgctag

SEQ ID NO: 22 - DNA, 1398 bp, synthetic construct
  source 1..1398: mol_type = other DNA; note = hu3F8-H3L3 heavy chain
atgggctggtcctgcatcatcctgttcctggtggccaccgccaccggccaggtgcagctggtcgaaagcgggcctggtctggtccagcctggtcgttctctgcgtctgacttgtgccgtgtccgggttctccgtcactaactacggagtgcactgggtcagacagccacctgggaagggtctggagtggctgggagtgatctgggcaggcggaattaccaactacaattccgccttcatgagcaggctgaccatctctaaggacaacagtaaaaatacagtgtatctgcagatgaattccctgagggccgaagatacagctgtctactattgcgcttctcggggcggtcactacggttacgctctggactactggggtcaggggactctggtcactgtcagcagcgcctccaccaagggcccatcggtcttccccctggcaccctcctccaagagcacctctgggggcacagcggccctgggctgcctggtcaaggactacttccccgaaccggtgacggtgtcgtggaactcaggcgccctgaccagcggcgtgcacaccttcccggccgtcctacagtcctcaggactctactccctcagcagcgtggtgaccgtgccctccagcagcttgggcacccagacctacatctgcaacgtgaatcacaagcccagcaacaccaaggtggacaagagagttgagcccaaatcttgtgacaaaactcacacatgcccaccgtgcccagcacctgaactcctggggggaccgtcagtcttcctcttccccccaaaacccaaggacaccctcatgatctcccggacccctgaggtcacatgcgtggtggtggacgtgagccacgaagaccctgaggtcaagttcaactggtacgtggacggcgtggaggtgcataatgccaagacaaagccgcgggaggagcagtacaacagcacgtaccgtgtggtcagcgtcctcaccgtcctgcaccaggactggctgaatggcaaggagtacaagtgcaaggtctccaacaaagccctcccagcccccatcgagaaaaccatctccaaagccaaagggcagccccgagaaccacaggtgtacaccctgcccccatcccgggatgagctgaccaagaaccaggtcagcctgacctgcctggtcaaaggcttctatcccagcgacatcgccgtggagtgggagagcaatgggcagccggagaacaactacaagaccacgcctcccgtgctggactccgacggctccttcttcctctacagcaagctcaccgtggacaagagcaggtggcagcaggggaacgtcttctcatgctccgtgatgcatgaggctctgcacaaccactacacgcagaagagcctctccctgtctccgggtaaatga

SEQ ID NO: 23 - protein, 518 aa, synthetic construct
  source 1..518: note = (hu3F8-LC) - (huOKT3-scFv)
EIVMTQTPATLSVSAGERVTITCKASQSVSNDVTWYQQKPGQAPRLLIYSASNRYSGVPARFSGSGYGTEFTFTISSVQSEDFAVYFCQQDYSSFGQGTKLEIKRTVAAPSVFIFPPSDEQLKSGTASVVCLLNNFYPREAKVQWKVDNALQSGNSQESVTEQDSKDSTYSLSSTLTLSKADYEKHKVYACEVTHQGLSSPVTKSFNRGECGGGGSGGGGSQVQLVQSGGGLTLSKADYEKHKVYACEVTHQGLSSPVTKSFNRGECGGGGSGGGGSQVQLVQSGGGVVQPGRSLRLSCKASGYTFTRYTMHWVRQAPGKCLEWIGYINPSRGYTNYNQKFKDRFTISRDNSKNTAFLQMDSLRPEDTGVYFCARYYDDHYCLDYWGQGTPVTVSSGGGGSGGGGSGGGGSDIQMTQSPSSLSASVGDRVTITCSASSSVSYMNWYQQTPGKAPKRWIYDTSKLASGVPSRFSGSGSGTDYTFTISSLQPEDIATYYCQQWSSNPFTFGCGTKLQITR

SEQ ID NO: 24 - protein, 524 aa, synthetic construct
  source 1..524: note = (hu3F8-LC) - (C8.2.5-scFv)
EIVMTQTPATLSVSAGERVTITCKASQSVSNDVTWYQQKPGQAPRLLIYSASNRYSGVPARFSGSGYGTEFTFTISSVQSEDFAVYFCQQDYSSFGQGTKLEIKRTVAAPSVFIFPPSDEQLKSGTASVVCLLNNFYPREAKVQWKVDNALQSGNSQESVTEQDSKDSTYSLSSTLTLSKADYEKHKVYACEVTHQGLSSPVTKSFNRGECGGGGSGGGGSASHVKLQESGPLTLSKADYEKHKVYACEVTHQGLSSPVTKSFNRGECGGGGSGGGGSASHVKLQESGPGLVQPSQSLSLTCTVSGFSLTDYGVHWVRQSPGKGLEWLGVIWSGGGTAYNTALISRLNIYRDNSKNQVFLEMNSLQAEDTAMYYCARRGSYPYNYFDAWGCGTTVTVSSGGGGSGGGGSGGGGSQAVVIQESALTTPPGETVTLTCGSSTGAVTASNYANWVQEKPDHCFTGLIGGHNNRPPGVPARFSGSLIGDKAALTIAGTQTEDEAIYFCALWYSDHWVIGGGTRLTVLG